European Patent Application EP 4 130 035 A1, published February 8, 2023. Title: ANTIBODY AND FUSION PROTEIN FOR TREATING CORONAVIRUSES AND USE THEREOF. Applicant: Bio-Thera Solutions, Ltd. The sequence listing filed with the application follows.

SEQUENCE LISTING (112 sequences)

SEQ ID NO: 1 - protein, 7 aa, Artificial Sequence
  Synthetic Peptide
FTFSSYA

SEQ ID NO: 2 - protein, 10 aa, Artificial Sequence
  Synthetic Peptide
AISGSGGSTY

SEQ ID NO: 3 - protein, 11 aa, Artificial Sequence
  Synthetic Peptide
ADYASTVYDYR

SEQ ID NO: 4 - protein, 11 aa, Artificial Sequence
  Synthetic Peptide
DRDPSASYYLD

SEQ ID NO: 5 - protein, 11 aa, Artificial Sequence
  Synthetic Peptide
GPLGFSAGGLP

SEQ ID NO: 6 - protein, 11 aa, Artificial Sequence
  Synthetic Peptide
GPFGIYDGYLP

SEQ ID NO: 7 - protein, 11 aa, Artificial Sequence
  Synthetic Peptide
GPYGYSPGYLP

SEQ ID NO: 8 - protein, 11 aa, Artificial Sequence
  Synthetic Peptide
GPFGFSDGYLP

SEQ ID NO: 9 - protein, 11 aa, Artificial Sequence
  Synthetic Peptide
HDDASPPGPDS

SEQ ID NO: 10 - protein, 11 aa, Artificial Sequence
  Synthetic Peptide
GPFGYSAGYLP

SEQ ID NO: 11 - protein, 11 aa, Artificial Sequence
  Synthetic Peptide
ADYASTVYDGR

SEQ ID NO: 12 - protein, 11 aa, Artificial Sequence
  Synthetic Peptide
HLGPTYGGYAR

SEQ ID NO: 13 - protein, 11 aa, Artificial Sequence
  Synthetic Peptide
GLYGYDLYLDR

SEQ ID NO: 14 - protein, 11 aa, Artificial Sequence
  Synthetic Peptide
ETSYDGYVTLA

SEQ ID NO: 15 - protein, 11 aa, Artificial Sequence
  Synthetic Peptide
HAEDSPPGPDS

SEQ ID NO: 16 - protein, 11 aa, Artificial Sequence
  Synthetic Peptide
GSYGYDLYLDR

SEQ ID NO: 17 - protein, 11 aa, Artificial Sequence
  Synthetic Peptide
GPFGYSDGYLP

SEQ ID NO: 18 - protein, 11 aa, Artificial Sequence
  Synthetic Peptide
DTGYFYATTLD

SEQ ID NO: 19 - protein, 11 aa, Artificial Sequence
  Synthetic Peptide
DLDPDAFYYLD

SEQ ID NO: 20 - protein, 11 aa, Artificial Sequence
  Synthetic Peptide
DRDPSAPYYLD

SEQ ID NO: 21 - protein, 11 aa, Artificial Sequence
  Synthetic Peptide
DRDPAAYYYLD

SEQ ID NO: 22 - protein, 11 aa, Artificial Sequence
  Synthetic Peptide
DRDPTAVYYLD

SEQ ID NO: 23 - protein, 11 aa, Artificial Sequence
  Synthetic Peptide
ESSYDGYVDLA

SEQ ID NO: 24 - protein, 11 aa, Artificial Sequence
  Synthetic Peptide
DRDPSAYYYLD

SEQ ID NO: 25 - protein, 11 aa, Artificial Sequence
  Synthetic Peptide
GPFGVSDGYLP

SEQ ID NO: 26 - protein, 11 aa, Artificial Sequence
  Synthetic Peptide
HPDESPPLPDR

SEQ ID NO: 27 - protein, 11 aa, Artificial Sequence
  Synthetic Peptide
GPYGYSAGYLP

SEQ ID NO: 28 - protein, 11 aa, Artificial Sequence
  Synthetic Peptide
HPTRYPAYTDP

SEQ ID NO: 29 - protein, 11 aa, Artificial Sequence
  Synthetic Peptide
GPFGYSSGYLP

SEQ ID NO: 30 - protein, 11 aa, Artificial Sequence
  Synthetic Peptide
ELYPGRFFPLY

SEQ ID NO: 31 - protein, 11 aa, Artificial Sequence
  Synthetic Peptide
HRYPRSYSPLS

SEQ ID NO: 32 - protein, 11 aa, Artificial Sequence
  Synthetic Peptide
DRDPSATYYLD

SEQ ID NO: 33 - protein, 11 aa, Artificial Sequence
  Synthetic Peptide
DTAYYYYTTLD

SEQ ID NO: 34 - protein, 11 aa, Artificial Sequence
  Synthetic Peptide
RVDLGLYYLDA

SEQ ID NO: 35 - protein, 11 aa, Artificial Sequence
  Synthetic Peptide
DTRYYYLSTLD

SEQ ID NO: 36 - protein, 12 aa, Artificial Sequence
  Synthetic Peptide
VPTRGIGRYDFL

SEQ ID NO: 37 - protein, 11 aa, Artificial Sequence
  Synthetic Peptide
DRARYNSYLVH

SEQ ID NO: 38 - protein, 11 aa, Artificial Sequence
  Synthetic Peptide
GPFGSSPGYLP

SEQ ID NO: 39 - protein, 6 aa, Artificial Sequence
  Synthetic Peptide
QGISSY

SEQ ID NO: 40 - protein, 3 aa, Artificial Sequence
  Synthetic Peptide
AAS

SEQ ID NO: 41 - protein, 7 aa, Artificial Sequence
  Synthetic Peptide
QQHYTTP

SEQ ID NO: 42 - protein, 28 aa, Artificial Sequence
  Synthetic Peptide
MAEVQLVESGGGLVQPGGSLRLSCTASG

SEQ ID NO: 43 - protein, 16 aa, Artificial Sequence
  Synthetic Peptide
MSWVRQAPGKGLEWVS

SEQ ID NO: 44 - protein, 39 aa, Artificial Sequence
  Synthetic Peptide
YADSVKGRFTISRDNSKNTLYLQMNSLRAEDTAVYYCAR

SEQ ID NO: 45 - protein, 13 aa, Artificial Sequence
  Synthetic Peptide
DYWGQGTLVTVSS

SEQ ID NO: 46 - protein, 124 aa, Artificial Sequence
  Synthetic Peptide
MAEVQLVESGGGLVQPGGSLRLSCTASGFTFSSYAMSWVRQAPGKGLEWVSAISGSGGSTYYADSVKGRFTISRDNSKNTLYLQMNSLRAEDTAVYYCARDRDPSASYYLDDYWGQGTLVTVSS

SEQ ID NO: 47 - protein, 124 aa, Artificial Sequence
  Synthetic Peptide
MAEVQLVESGGGLVQPGGSLRLSCTASGFTFSSYAMSWVRQAPGKGLEWVSAISGSGGSTYYADSVKGRFTISRDNSKNTLYLQMNSLRAEDTAVYYCARGPFGYSAGYLPDYWGQGTLVTVSS

SEQ ID NO: 48 - protein, 124 aa, Artificial Sequence
  Synthetic Peptide
MAEVQLVESGGGLVQPGGSLRLSCTASGFTFSSYAMSWVRQAPGKGLEWVSAISGSGGSTYYADSVKGRFTISRDNSKNTLYLQMNSLRAEDTAVYYCARHLGPTYGGYARDYWGQGTLVTVSS

SEQ ID NO: 49 - protein, 124 aa, Artificial Sequence
  Synthetic Peptide
MAEVQLVESGGGLVQPGGSLRLSCTASGFTFSSYAMSWVRQAPGKGLEWVSAISGSGGSTYYADSVKGRFTISRDNSKNTLYLQMNSLRAEDTAVYYCARETSYDGYVTLADYWGQGTLVTVSS

SEQ ID NO: 50 - protein, 107 aa, Artificial Sequence
  Synthetic Peptide
DIQMTQSPSSLSASVGDRVTITCRASQGISSYLAWYQQKPGKAPKLLIYAASSLQSGVPSRFSGSGSGTDFTLTISSLQPEDFATYYCQQHYTTPPTFGQGTKVEIK

SEQ ID NO: 51 - protein, 330 aa, Artificial Sequence
  Synthetic Peptide
ASTKGPSVFPLAPSSKSTSGGTAALGCLVKDYFPEPVTVSWNSGALTSGVHTFPAVLQSSGLYSLSSVVTVPSSSLGTQTYICNVNHKPSNTKVDKKVEPKSCDKTHTCPPCPAPELLGGPSVFLFPPKPKDTLYITREPEVTCVVVDVSHEDPEVKFNWYVDGVEVHNAKTKPREEQYASTYRVVSVLTVLHQDWLNGKEYKCKVSNKALPAPIEKTISKAKGQPREPQVYTLPPSRDELTKNQVSLTCLVKGFYPSDIAVEWESNGQPENNYKTTPPVLDSDGSFFLYSKLTVDKSRWQQGNVFSCSVMHEALHNHYTQKSLSLSPGK

SEQ ID NO: 52 - protein, 107 aa, Artificial Sequence [sequence omitted]

SEQ ID NO: 53 - protein, 454 aa, Artificial Sequence
  Synthetic Peptide
MAEVQLVESGGGLVQPGGSLRLSCTASGFTFSSYAMSWVRQAPGKGLEWVSAISGSGGSTYYADSVKGRFTISRDNSKNTLYLQMNSLRAEDTAVYYCARDRDPSASYYLDDYWGQGTLVTVSSASTKGPSVFPLAPSSKSTSGGTAALGCLVKDYFPEPVTVSWNSGALTSGVHTFPAVLQSSGLYSLSSVVTVPSSSLGTQTYICNVNHKPSNTKVDKKVEPKSCDKTHTCPPCPAPELLGGPSVFLFPPKPKDTLYITREPEVTCVVVDVSHEDPEVKFNWYVDGVEVHNAKTKPREEQYASTYRVVSVLTVLHQDWLNGKEYKCKVSNKALPAPIEKTISKAKGQPREPQVYTLPPSRDELTKNQVSLTCLVKGFYPSDIAVEWESNGQPENNYKTTPPVLDSDGSFFLYSKLTVDKSRWQQGNVFSCSVMHEALHNHYTQKSLSLSPGK

SEQ ID NO: 54 - protein, 454 aa, Artificial Sequence
  Synthetic Peptide
MAEVQLVESGGGLVQPGGSLRLSCTASGFTFSSYAMSWVRQAPGKGLEWVSAISGSGGSTYYADSVKGRFTISRDNSKNTLYLQMNSLRAEDTAVYYCARGPFGYSAGYLPDYWGQGTLVTVSSASTKGPSVFPLAPSSKSTSGGTAALGCLVKDYFPEPVTVSWNSGALTSGVHTFPAVLQSSGLYSLSSVVTVPSSSLGTQTYICNVNHKPSNTKVDKKVEPKSCDKTHTCPPCPAPELLGGPSVFLFPPKPKDTLYITREPEVTCVVVDVSHEDPEVKFNWYVDGVEVHNAKTKPREEQYASTYRVVSVLTVLHQDWLNGKEYKCKVSNKALPAPIEKTISKAKGQPREPQVYTLPPSRDELTKNQVSLTCLVKGFYPSDIAVEWESNGQPENNYKTTPPVLDSDGSFFLYSKLTVDKSRWQQGNVFSCSVMHEALHNHYTQKSLSLSPGK

SEQ ID NO: 55 - protein, 454 aa, Artificial Sequence
  Synthetic Peptide
MAEVQLVESGGGLVQPGGSLRLSCTASGFTFSSYAMSWVRQAPGKGLEWVSAISGSGGSTYYADSVKGRFTISRDNSKNTLYLQMNSLRAEDTAVYYCARHLGPTYGGYARDYWGQGTLVTVSSASTKGPSVFPLAPSSKSTSGGTAALGCLVKDYFPEPVTVSWNSGALTSGVHTFPAVLQSSGLYSLSSVVTVPSSSLGTQTYICNVNHKPSNTKVDKKVEPKSCDKTHTCPPCPAPELLGGPSVFLFPPKPKDTLYITREPEVTCVVVDVSHEDPEVKFNWYVDGVEVHNAKTKPREEQYASTYRVVSVLTVLHQDWLNGKEYKCKVSNKALPAPIEKTISKAKGQPREPQVYTLPPSRDELTKNQVSLTCLVKGFYPSDIAVEWESNGQPENNYKTTPPVLDSDGSFFLYSKLTVDKSRWQQGNVFSCSVMHEALHNHYTQKSLSLSPGK

SEQ ID NO: 56 - protein, 454 aa, Artificial Sequence
  Synthetic Peptide
MAEVQLVESGGGLVQPGGSLRLSCTASGFTFSSYAMSWVRQAPGKGLEWVSAISGSGGSTYYADSVKGRFTISRDNSKNTLYLQMNSLRAEDTAVYYCARETSYDGYVTLADYWGQGTLVTVSSASTKGPSVFPLAPSSKSTSGGTAALGCLVKDYFPEPVTVSWNSGALTSGVHTFPAVLQSSGLYSLSSVVTVPSSSLGTQTYICNVNHKPSNTKVDKKVEPKSCDKTHTCPPCPAPELLGGPSVFLFPPKPKDTLYITREPEVTCVVVDVSHEDPEVKFNWYVDGVEVHNAKTKPREEQYASTYRVVSVLTVLHQDWLNGKEYKCKVSNKALPAPIEKTISKAKGQPREPQVYTLPPSRDELTKNQVSLTCLVKGFYPSDIAVEWESNGQPENNYKTTPPVLDSDGSFFLYSKLTVDKSRWQQGNVFSCSVMHEALHNHYTQKSLSLSPGK

SEQ ID NO: 57 - protein, 214 aa, Artificial Sequence
  Synthetic Peptide
DIQMTQSPSSLSASVGDRVTITCRASQGISSYLAWYQQKPGKAPKLLIYAASSLQSGVPSRFSGSGSGTDFTLTISSLQPEDFATYYCQQHYTTPPTFGQGTKVEIKRTVAAPSVFIFPPSDEQLKSGTASVVCLLNNFYPREAKVQWKVDNALQSGNSQESVTEQDSKDSTYSLSSTLTLSKADYEKHKVYACEVTHQGLSSPVTKSFNRGEC

SEQ ID NO: 58 - protein, 36 aa, Artificial Sequence
  Synthetic Peptide
DISGINASVVNIQKEIDRLNEVAKNLNESLIDLQEL

SEQ ID NO: 59 - protein, 20 aa, Artificial Sequence
  Synthetic Peptide
GGGGSGGGGSGGGGSGGGGS

SEQ ID NO: 60 - protein, 5 aa, Artificial Sequence
  Synthetic Peptide
SYAMS

SEQ ID NO: 61 - protein, 17 aa, Artificial Sequence
  Synthetic Peptide
AISGSGGSTYYADSVKG

SEQ ID NO: 62 - protein, 13 aa, Artificial Sequence
  Synthetic Peptide
ADYASTVYDYRDY

SEQ ID NO: 63 - protein, 13 aa, Artificial Sequence
  Synthetic Peptide
DRDPSASYYLDDY

SEQ ID NO: 64 - protein, 13 aa, Artificial Sequence
  Synthetic Peptide
GPLGFSAGGLPDY

SEQ ID NO: 65 - protein, 13 aa, Artificial Sequence
  Synthetic Peptide
GPFGIYDGYLPDY

SEQ ID NO: 66 - protein, 13 aa, Artificial Sequence
  Synthetic Peptide
GPYGYSPGYLPDY

SEQ ID NO: 67 - protein, 13 aa, Artificial Sequence
  Synthetic Peptide
GPFGFSDGYLPDY

SEQ ID NO: 68 - protein, 13 aa, Artificial Sequence
  Synthetic Peptide
HDDASPPGPDSDY

SEQ ID NO: 69 - protein, 13 aa, Artificial Sequence
  Synthetic Peptide
GPFGYSAGYLPDY

SEQ ID NO: 70 - protein, 13 aa, Artificial Sequence
  Synthetic Peptide
ADYASTVYDGRDY

SEQ ID NO: 71 - protein, 13 aa, Artificial Sequence
  Synthetic Peptide
HLGPTYGGYARDY

SEQ ID NO: 72 - protein, 13 aa, Artificial Sequence
  Synthetic Peptide
GLYGYDLYLDRDY

SEQ ID NO: 73 - protein, 13 aa, Artificial Sequence
  Synthetic Peptide
ETSYDGYVTLADY

SEQ ID NO: 74 - protein, 13 aa, Artificial Sequence
  Synthetic Peptide
HAEDSPPGPDSDY

SEQ ID NO: 75 - protein, 13 aa, Artificial Sequence
  Synthetic Peptide
GSYGYDLYLDRDY

SEQ ID NO: 76 - protein, 13 aa, Artificial Sequence
  Synthetic Peptide
GPFGYSDGYLPDY

SEQ ID NO: 77 - protein, 13 aa, Artificial Sequence
  Synthetic Peptide
DTGYFYATTLDDY

SEQ ID NO: 78 - protein, 13 aa, Artificial Sequence
  Synthetic Peptide
DLDPDAFYYLDDY

SEQ ID NO: 79 - protein, 13 aa, Artificial Sequence
  Synthetic Peptide
DRDPSAPYYLDDY

SEQ ID NO: 80 - protein, 13 aa, Artificial Sequence
  Synthetic Peptide
DRDPAAYYYLDDY

SEQ ID NO: 81 - protein, 13 aa, Artificial Sequence
  Synthetic Peptide
DRDPTAVYYLDDY

SEQ ID NO: 82 - protein, 13 aa, Artificial Sequence
  Synthetic Peptide
ESSYDGYVDLADY

SEQ ID NO: 83 - protein, 13 aa, Artificial Sequence
  Synthetic Peptide
DRDPSAYYYLDDY

SEQ ID NO: 84 - protein, 13 aa, Artificial Sequence
  Synthetic Peptide
GPFGVSDGYLPDY

SEQ ID NO: 85 - protein, 13 aa, Artificial Sequence
  Synthetic Peptide
HPDESPPLPDRDY

SEQ ID NO: 86 - protein, 13 aa, Artificial Sequence
  Synthetic Peptide
GPYGYSAGYLPDY

SEQ ID NO: 87 - protein, 13 aa, Artificial Sequence
  Synthetic Peptide
HPTRYPAYTDPDY

SEQ ID NO: 88 - protein, 13 aa, Artificial Sequence
  Synthetic Peptide
GPFGYSSGYLPDY

SEQ ID NO: 89 - protein, 13 aa, Artificial Sequence
  Synthetic Peptide
ELYPGRFFPLYDY

SEQ ID NO: 90 - protein, 13 aa, Artificial Sequence
  Synthetic Peptide
HRYPRSYSPLSDY

SEQ ID NO: 91 - protein, 13 aa, Artificial Sequence
  Synthetic Peptide
DRDPSATYYLDDY

SEQ ID NO: 92 - protein, 13 aa, Artificial Sequence
  Synthetic Peptide
DTAYYYYTTLDDY

SEQ ID NO: 93 - protein, 13 aa, Artificial Sequence
  Synthetic Peptide
RVDLGLYYLDADY

SEQ ID NO: 94 - protein, 13 aa, Artificial Sequence
  Synthetic Peptide
DTRYYYLSTLDDY

SEQ ID NO: 95 - protein, 14 aa, Artificial Sequence
  Synthetic Peptide
VPTRGIGRYDFLDY

SEQ ID NO: 96 - protein, 13 aa, Artificial Sequence
  Synthetic Peptide
DRARYNSYLVHDY

SEQ ID NO: 97 - protein, 13 aa, Artificial Sequence
  Synthetic Peptide
GPFGSSPGYLPDY

SEQ ID NO: 98 - protein, 11 aa, Artificial Sequence
  Synthetic Peptide
RASQGISSYLA

SEQ ID NO: 99 - protein, 7 aa, Artificial Sequence
  Synthetic Peptide
AASSLQS

SEQ ID NO: 100 - protein, 9 aa, Artificial Sequence
  Synthetic Peptide
QQHYTTPPT

SEQ ID NO: 101 - protein, 30 aa, Artificial Sequence
  Synthetic Peptide
EVQLVESGGGLVQPGGSLRLSCTASGFTFS

SEQ ID NO: 102 - protein, 14 aa, Artificial Sequence
  Synthetic Peptide
WVRQAPGKGLEWVS

SEQ ID NO: 103 - protein, 32 aa, Artificial Sequence
  Synthetic Peptide
RFTISRDNSKNTLYLQMNSLRAEDTAVYYCAR

SEQ ID NO: 104 - protein, 11 aa, Artificial Sequence
  Synthetic Peptide
WGQGTLVTVSS

SEQ ID NO: 105 - protein, 11 aa, Artificial Sequence
  Synthetic Peptide
GPFGIDDAYLP

SEQ ID NO: 106 - protein, 13 aa, Artificial Sequence
  Synthetic Peptide
GPFGIDDAYLPDY

SEQ ID NO: 107 - protein, 122 aa, Artificial Sequence
  Synthetic Peptide
EVQLVESGGGLVQPGGSLRLSCTASGFTFSSYAMSWVRQAPGKGLEWVSAISGSGGSTYYADSVKGRFTISRDNSKNTLYLQMNSLRAEDTAVYYCARGPFGIDDAYLPDYWGQGTLVTVSS

SEQ ID NO: 108 - protein, 452 aa, Artificial Sequence
  Synthetic Peptide
EVQLVESGGGLVQPGGSLRLSCTASGFTFSSYAMSWVRQAPGKGLEWVSAISGSGGSTYYADSVKGRFTISRDNSKNTLYLQMNSLRAEDTAVYYCARGPFGIDDAYLPDYWGQGTLVTVSSASTKGPSVFPLAPSSKSTSGGTAALGCLVKDYFPEPVTVSWNSGALTSGVHTFPAVLQSSGLYSLSSVVTVPSSSLGTQTYICNVNHKPSNTKVDKKVEPKSCDKTHTCPPCPAPELLGGPSVFLFPPKPKDTLYITREPEVTCVVVDVSHEDPEVKFNWYVDGVEVHNAKTKPREEQYASTYRVVSVLTVLHQDWLNGKEYKCKVSNKALPAPIEKTISKAKGQPREPQVYTLPPSRDELTKNQVSLTCLVKGFYPSDIAVEWESNGQPENNYKTTPPVLDSDGSFFLYSKLTVDKSRWQQGNVFSCSVMHEALHNHYTQKSLSLSPGK

SEQ ID NO: 109 - DNA, 1518 bp, Artificial Sequence
  Synthetic Oligonucleotide
gaagtgcaattggtggaaagcggcggcggcctggtgcagccgggcggcagcctgcgcctgagctgcgcggcgtccggatttacctttagcagctatgcgatgagctgggtgcgccaggcaccgggcaaaggcctcgaatgggtgagcgcgattagcggcagcggcggcagcacctattatgcggatagcgtgaaaggccgctttaccattagccgcgataattcgaaaaacaccctgtatctgcaaatgaacagcctgcgtgcggaagatactgcagtgtattattgcgcgcgtggtccgttcggtatcgacgacgcttacctgccggattattggggccaaggcaccctggtgacggtgagcagcgcctctaccaagggcccctctgtgtttcctctggctccctccagcaagtctacctctggtggaacagctgccctgggctgcctggtcaaggattactttcctgagcctgtcaccgtgtcctggaactctggcgctctgacatctggcgtgcacacctttccagctgtgctccagtcctccggcctgtactctctgtcctctgtcgtgaccgtgccttctagctctctgggcacccagacctacatctgcaatgtgaaccacaagccttccaacaccaaggtggacaagaaggtggaacccaagtcctgcgacaagacccacacctgtcctccatgtcctgctccagaactgctcggcggaccttccgtgttcctgtttcctccaaagcctaaggacaccctgatgatctctcggacccctgaagtgacctgcgtggtggtggatgtgtctcacgaagatcccgaagtgaagttcaactggtacgtggacggcgtggaagtgcacaacgccaagaccaagcctagagaggaacagtacaactccacctacagagtggtgtccgtgctgaccgtgctgcaccaggattggctgaacggcaaagagtacaagtgcaaggtgtccaacaaggccctgcctgctcctatcgaaaagaccatctccaaggccaagggccagcctagggaaccccaggtttacaccttgcctccatctcgggacgagctgaccaagaaccaggtgtccctgacctgtctcgtgaagggcttctacccctccgacatcgccgtggaatgggagtctaatggccagcctgagaacaactacaagacaacccctcctgtgctggactccgacggctcattcttcctgtactccaagctgacagtggacaagtccagatggcagcagggcaacgtgttctcctgctccgtgatgcacgaggccctgcacaatcactacacccagaagtccctgtctctgtcccctggaggaggaggctccggaggaggcggaagcggaggaggaggatctggcggcggcggatctgacatctctggcatcaatgcctctgtggtgaacatccagaaggagattgacagactgaatgaggtggctaagaacctgaatgagtccctgattgacctccaagaactg

SEQ ID NO: 110 - DNA, 642 bp, Artificial Sequence
  Synthetic Oligonucleotide
gatatccagatgacccagtcccccagctccctgagcgctagcgtgggcgaccgggtgaccatcacctgcagggcctcccagggcatcagctcctacctggcttggtatcagcagaagcctggcaaggcccctaagctgctgatctatgccgcttcctccctgcagtccggcgtgccttccaggttcagcggctccggcagcggcaccgacttcaccctgaccatctcctccctgcagcctgaggacttcgccacctattattgccagcagcactataccacccctcctacctttggccagggcaccaaggtggagatcaagcgtacggtggctgcaccatctgtcttcatcttcccgccatctgatgagcagttgaaatctggaactgcctctgttgtgtgcctgctgaataacttctatcccagagaggccaaagtacagtggaaggtggataacgccctccaatcgggtaactcccaggagagtgtcacagagcaggacagcaaggacagcacctacagcctcagcagcaccctgacgctgagcaaagcagactacgagaaacacaaagtctacgcctgcgaagtcacccatcagggcctgagctcgcccgtcacaaagagcttcaacaggggagagtgt

SEQ ID NO: 111 - protein, 506 aa, Artificial Sequence
  Synthetic Peptide
EVQLVESGGGLVQPGGSLRLSCTASGFTFSSYAMSWVRQAPGKGLEWVSAISGSGGSTYYADSVKGRFTISRDNSKNTLYLQMNSLRAEDTAVYYCARGPFGIDDAYLPDYWGQGTLVTVSSASTKGPSVFPLAPSSKSTSGGTAALGCLVKDYFPEPVTVSWNSGALTSGVHTFPAVLQSSGLYSLSSVVTVPSSSLGTQTYICNVNHKPSNTKVDKKVEPKSCDKTHTCPPCPAPELLGGPSVFLFPPKPKDTLYITREPEVTCVVVDVSHEDPEVKFNWYVDGVEVHNAKTKPREEQYASTYRVVSVLTVLHQDWLNGKEYKCKVSNKALPAPIEKTISKAKGQPREPQVYTLPPSRDELTKNQVSLTCLVKGFYPSDIAVEWESNGQPENNYKTTPPVLDSDGSFFLYSKLTVDKSRWQQGNVFSCSVMHEALHNHYTQKSLSLSPGGGGSGGGGSGGGGSGGGGSDISGINASVVNIQKEIDRLNEVAKNLNESLIDLQEL

SEQ ID NO: 112 - protein, 214 aa, Artificial Sequence; identical to SEQ ID NO: 57
  Synthetic Peptide